European Patent Specification EP 3 438 123 B1, published June 3, 2026. Title: RECEPTOR. Applicant: Autolus Ltd. The sequence listing filed with the application follows.

SEQUENCE LISTING (55 sequences)

SEQ ID NO: 1 - protein, 86 aa, Artificial Sequence
  endodomain derived from IL-2 receptor common gamma-chain
ERTMPRIPTLKNLEDLVTEYHGNFSAWSGVSKGLAESLQPDYSERLCLVSEIPPKGGALGEGPGASPCNQHSPYWAPPCYTLKPET

SEQ ID NO: 2 - protein, 286 aa, Artificial Sequence
  endodomain derived from IL-2 receptor common beta-chain
NCRNTGPWLKKVLKCNTPDPSKFFSQLSSEHGGDVQKWLSSPFPSSSFSPGGLAPEISPLEVLERDKVTQLLLQQDKVPEPASLSSNHSLTSCFTNQGYFFFHLPDALEIEACQVYFTYDPYSEEDPDEGVAGAPTGSSPQPLQPLSGEDDAYCTFPSRDDLLLFSPSLLGGPSPPSTAPGGSGAGEERMPPSLQERVPRDWDPQPLGPPTPGVPDLVDFQPPPELVLREAGEEVPDAGPREGVSFPWSRPPGQGEFRALNARLPLNTDAYLSLQELQGQDPTHLV

SEQ ID NO: 3 - protein, 195 aa, Artificial Sequence
  endodomain derived from IL-7 receptor alpha-chain
KKRIKPIVWPSLPDHKKTLEHLCKKPRKNLNVSFNPESFLDCQIHRVDDIQARDEVEGFLQDTFPQQLEESEKQRLGGDVQSPNCPSEDVVITPESFGRDSSLTCLAGNVSACDAPILSSSRSLDCRESGKNGPHVYQDLLLSLGTTNSTLPPPFSLQSGILTLNPVAQGQPILTSLGSNQEEAYVTMSSFYQNQ

SEQ ID NO: 4 - protein, 234 aa, Artificial Sequence
  hinge-CH2CH3 of human IgG1
AEPKSPDKTHTCPPCPAPPVAGPSVFLFPPKPKDTLMIARTPEVTCVVVDVSHEDPEVKFNWYVDGVEVHNAKTKPREEQYNSTYRVVSVLTVLHQDWLNGKEYKCKVSNKALPAPIEKTISKAKGQPREPQVYTLPPSRDELTKNQVSLTCLVKGFYPSDIAVEWESNGQPENNYKTTPPVLDSDGSFFLYSKLTVDKSRWQQGNVFSCSVMHEALHNHYTQKSLSLSPGKKD

SEQ ID NO: 5 - protein, 46 aa, Artificial Sequence
  human CD8 stalk
TTTPAPRPPTPAPTIASQPLSLRPEACRPAAGGAVHTRGLDFACDI

SEQ ID NO: 6 - protein, 20 aa, Artificial Sequence
  human IgG1 hinge
AEPKSPDKTHTCPPCPKDPK

SEQ ID NO: 7 - protein, 21 aa, Artificial Sequence
  transmembrane derived from human common gamma chain
VVISVGSMGLIISLLCVYFWL

SEQ ID NO: 8 - protein, 25 aa, Artificial Sequence
  transmembrane derived from human IL-2Rbeta
IPWLGHLLVGLSGAFGFIILVYLLI

SEQ ID NO: 9 - protein, 25 aa, Artificial Sequence
  transmembrane derived from human IL-7Ralpha
PILLTISILSFFSVALLVILACVLW

SEQ ID NO: 10 - protein, 22 aa, Artificial Sequence
  transmembrane derived from human IL-15Ralpha
AISTSTVLLCGLSAVSLLACYL

SEQ ID NO: 11 - protein, 118 aa, Artificial Sequence
  sequence of 5D3D11 VH
QVQLQQSGPELVKPGASVKISCKVSGYAISSSWMNWVKQRPGQGLEWIGRIYPGDGDTKYNGKFKDKATLTVDKSSSTAYMQLSSLTSVDSAVYFCARDGYRYYFDYWGQGTSVTVSS

SEQ ID NO: 12 - protein, 112 aa, Artificial Sequence
  sequence of 5D3D11 VL
DIVMTQTAPSVFVTPGESVSISCRSSKSLLHSNGNTYLYWFLQRPGQSPQLLIYRMSNLASGVPDRFSGSGSGTDFTLRISRVEAEDVGVYYCMQHLEYPVTFGAGTKVEIK

SEQ ID NO: 13 - protein, 117 aa, Artificial Sequence
  sequence of 5D5A5 VH
QVQLQQSGAELAKPGASVKMSCKTSGYSFSSYWMHWVKQRPGQGLEWIGYINPSTGYTENNQKFKDKVTLTADKSSNTAYMQLNSLTSEDSAVYYCARSGRLYFDVWGAGTTVTVSS

SEQ ID NO: 14 - protein, 111 aa, Artificial Sequence
  sequence of 5D5A5 VL
DIVLTQSPPSLAVSLGQRATISCRASESIDLYGFTFMHWYQQKPGQPPKILIYRASNLESGIPARFSGSGSRTDFTLTINPVEADDVATYYCQQTHEDPYTFGGGTKLEIK

SEQ ID NO: 15 - protein, 248 aa, Artificial Sequence
  ScFv based on 5D5A5
QVQLQQSGAELAKPGASVKMSCKTSGYSFSSYWMHWVKQRPGQGLEWIGYINPSTGYTENNQKFKDKVTLTADKSSNTAYMQLNSLTSEDSAVYYCARSGRLYFDVWGAGTTVTVSSGGGGSGGGGSGGGGSGGGGSDIVLTQSPPSLAVSLGQRATISCRASESIDLYGFTFMHWYQQKPGQPPKILIYRASNLESGIPARFSGSGSRTDFTLTINPVEADDVATYYCQQTHEDPYTFGGGTKLEIK

SEQ ID NO: 16 - protein, 250 aa, Artificial Sequence
  ScFv based on 5D3D11
QVQLQQSGPELVKPGASVKISCKVSGYAISSSWMNWVKQRPGQGLEWIGRIYPGDGDTKYNGKFKDKATLTVDKSSSTAYMQLSSLTSVDSAVYFCARDGYRYYFDYWGQGTSVTVSSGGGGSGGGGSGGGGSGGGGSDIVMTQTAPSVFVTPGESVSISCRSSKSLLHSNGNTYLYWFLQRPGQSPQLLIYRMSNLASGVPDRFSGSGSGTDFTLRISRVEAEDVGVYYCMQHLEYPVTFGAGTKVEIK

SEQ ID NO: 17 - protein, 356 aa, Artificial Sequence
  sequence of CXCR4
MSIPLPLLQIYTSDNYTEEMGSGDYDSMKEPCFREENANFNKIFLPTIYSIIFLTGIVGNGLVILVMGYQKKLRSMTDKYRLHLSVADLLFVITLPFWAVDAVANWYFGNFLCKAVHVIYTVNLYSSVLILAFISLDRYLAIVHATNSQRPRKLLAEKVVYVGVWIPALLLTIPDFIFANVSEADDRYICDRFYPNDLWVVVFQFQHIMVGLILPGIVILSCYCIIISKLSHSKGHQKRKALKTTVILILAFFACWLPYYIGISIDSFILLEIIKQGCEFENTVHKWISITEALAFFHCCLNPILYAFLGAKFKTSAQHALTSVSRGSSLKILSKGKRGGHSSVSTESESSSFHSS

SEQ ID NO: 18 - protein, 374 aa, Artificial Sequence
  sequence of cell surface receptor CCR2
MLSTSRSRFIRNTNESGEEVTTFFDYDYGAPCHKFDVKQIGAQLLPPLYSLVFIFGFVGNMLVVLILINCKKLKCLTDIYLLNLAISDLLFLITLPLWAHSAANEWVFGNAMCKLFTGLYHIGYFGGIFFIILLTIDRYLAIVHAVFALKARTVTFGVVTSVITWLVAVFASVPGIIFTKCQKEDSVYVCGPYFPRGWNNFHTIMRNILGLVLPLLIMVICYSGILKTLLRCRNEKKRHRAVRVIFTIMIVYFLFWTPYNIVILLNTFQEFFGLSNCESTSQLDQATQVTETLGMTHCCINPIIYAFVGEKFRSLFHIALGCRIAPLQKPVCGGPGVRPGKNVKVTTQGLLDGRGKGKSIGRAPEASLQDKEGA

SEQ ID NO: 19 - protein, 360 aa, Artificial Sequence
  sequence of cell surface receptor CCR4
MNPTDIADTTLDESIYSNYYLYESIPKPCTKEGIKAFGELFLPPLYSLVFVFGLLGNSVVVLVLFKYKRLRSMTDVYLLNLAISDLLFVFSLPFWGYYAADQWVFGLGLCKMISWMYLVGFYSGIFFVMLMSIDRYLAIVHAVFSLRARTLTYGVITSLATWSVAVFASLPGFLFSTCYTERNHTYCKTKYSLNSTTWKVLSSLEINILGLVIPLGIMLFCYSMIIRTLQHCKNEKKNKAVKMIFAVVVLFLGFWTPYNIVLFLETLVELEVLQDCTFERYLDYAIQATETLAFVHCCLNPIIYFFLGEKFRKYILQLFKTCRGLFVLCQYCGLLQIYSADTPSSSYTQSTMDHDLHDAL

SEQ ID NO: 20 - protein, 238 aa, Artificial Sequence
  scFv based on J591
EVQLQQSGPELKKPGTSVRISCKTSGYTFTEYTIHWVKQSHGKSLEWIGNINPNNGGTTYNQKFEDKATLTVDKSSSTAYMELRSLTSEDSAVYYCAAGWNFDYWGQGTTLTVSSGGGGSGGGGSGGGGSDIVMTQSHKFMSTSVGDRVSIICKASQDVGTAVDWYQQKPGQSPKLLIYWASTRHTGVPDRFTGSGSGTDFTLTITNVQSEDLADYFCQQYNSYPLTFGAGTMLDLKR

SEQ ID NO: 21 - protein, 21 aa, Artificial Sequence
  signal peptide derived from TCR beta chain
MGTSLLCWMALCLLGADHADG

SEQ ID NO: 22 - protein, 21 aa, Artificial Sequence
  signal peptide derived from IgG1
MSLPVTALLLPLALLLHAARP

SEQ ID NO: 23 - protein, 20 aa, Artificial Sequence
  signal peptide derived from CD8a
MAVPTQVLGLLLLWLTDARC

SEQ ID NO: 24 - protein, 112 aa, Artificial Sequence
  CD3 Z endodomain
RVKFSRSADAPAYQQGQNQLYNELNLGRREEYDVLDKRRGRDPEMGGKPRRKNPQEGLYNELQKDKMAEAYSEIGMKGERRRGKGHDGLYQGLSTATKDTYDALHMQALPPR

SEQ ID NO: 25 - protein, 152 aa, Artificial Sequence
  CD28 and CD3 Zeta endodomains
SKRSRLLHSDYMNMTPRRPGPTRKHYQPYAPPRDFAAYRSRVKFSRSADAPAYQQGQNQLYNELNLGRREEYDVLDKRRGRDPEMGGKPRRKNPQEGLYNELQKDKMAEAYSEIGMKGERRRGKGHDGLYQGLSTATKDTYDALHMQALPPR

SEQ ID NO: 26 - protein, 188 aa, Artificial Sequence
  CD28, OX40 and CD3 Zeta endodomains
SKRSRLLHSDYMNMTPRRPGPTRKHYQPYAPPRDFAAYRSRDQRLPPDAHKPPGGGSFRTPIQEEQADAHSTLAKIRVKFSRSADAPAYQQGQNQLYNELNLGRREEYDVLDKRRGRDPEMGGKPRRKNPQEGLYNELQKDKMAEAYSEIGMKGERRRGKGHDGLYQGLSTATKDTYDALHMQALPPR

SEQ ID NO: 27 - protein, 38 aa, Artificial Sequence
  ICOS endodomain
CWLTKKKYSSSVHDPNGEYMFMRAVNTAKKSRLTDVTL

SEQ ID NO: 28 - protein, 48 aa, Artificial Sequence
  CD27 endodomain
QRRKYRSNKGESPVEPAEPCHYSCPREEEGSTIPIQEDYRKPEPACSP

SEQ ID NO: 29 - protein, 111 aa, Artificial Sequence
  BTLA endodomain
RRHQGKQNELSDTAGREINLVDAHLKSEQTEASTRQNSQVLLSETGIYDNDPDLCFRMQEGSEVYSNPCLEENKPGIVYASLNHSVIGPNSRLARNVKEAPTEYASICVRS

SEQ ID NO: 30 - protein, 188 aa, Artificial Sequence
  CD30 endodomain
HRRACRKRIRQKLHLCYPVQTSQPKLELVDSRPRRSSTQLRSGASVTEPVAEERGLMSQPLMETCHSVGAAYLESLPLQDASPAGGPSSPRDLPEPRVSTEHTNNKIEKIYIMKADTVIVGTVKAELPEGRGLAGPAEPELEEELEADHTPHYPEQETEPPLGSCSDVMLSVEEEGKEDPLPTAASGK

SEQ ID NO: 31 - protein, 58 aa, Artificial Sequence
  GITR endodomain
QLGLHIWQLRSQCMWPRETQLLLEVPPSTEDARSCQFPEEERGERSAEEKGRLGDLWV

SEQ ID NO: 32 - protein, 60 aa, Artificial Sequence
  HVEM endodomain
CVKRRKPRGDVVKVIVSVQRKRQEAEGEATVIEALQAPPDVTTVAVEETIPSFTGRSPNH

SEQ ID NO: 33 - protein, 20 aa, Artificial Sequence
  cleavage site, 2A-like sequence
YHADYYKQRLIHDVEMNPGP

SEQ ID NO: 34 - protein, 20 aa, Artificial Sequence
  cleavage site, 2A-like sequence
HYAGYFADLLIHDIETNPGP

SEQ ID NO: 35 - protein, 20 aa, Artificial Sequence
  cleavage site, 2A-like sequence
QCTNYALLKLAGDVESNPGP

SEQ ID NO: 36 - protein, 19 aa, Artificial Sequence
  cleavage site, 2A-like sequence
ATNFSLLKQAGDVEENPGP

SEQ ID NO: 37 - protein, 19 aa, Artificial Sequence
  cleavage site, 2A-like sequence
AARQMLLLLSGDVETNPGP

SEQ ID NO: 38 - protein, 20 aa, Artificial Sequence
  cleavage site, 2A-like sequence
RAEGRGSLLTCGDVEENPGP

SEQ ID NO: 39 - protein, 20 aa, Artificial Sequence
  cleavage site, 2A-like sequence
TRAEIEDELIRAGIESNPGP

SEQ ID NO: 40 - protein, 20 aa, Artificial Sequence
  cleavage site, 2A-like sequence
TRAEIEDELIRADIESNPGP

SEQ ID NO: 41 - protein, 20 aa, Artificial Sequence
  cleavage site, 2A-like sequence
AKFQIDKILISGDVELNPGP

SEQ ID NO: 42 - protein, 20 aa, Artificial Sequence
  cleavage site, 2A-like sequence
SSIIRTKMLVSGDVEENPGP

SEQ ID NO: 43 - protein, 20 aa, Artificial Sequence
  cleavage site, 2A-like sequence
CDAQRQKLLLSGDIEQNPGP

SEQ ID NO: 44 - protein, 20 aa, Artificial Sequence
  cleavage site, 2A-like sequence
YPIDFGGFLVKADSEFNPGP

SEQ ID NO: 45 - protein, 1722 aa, Artificial Sequence
  fusion construct with IL-2R beta chain
MSLPVTALLLPLALLLHAAEVQLQQSGPELKKPGTSVRISCKTSGYTFTEYTIHWVKQSHGKSLEWIGNINPNNGGTTYNQKFEDKATLTVDKSSSTAYMELRSLTSEDSAVYYCAAGWNFDYWGQGTTLTVSSGGGGSGGGGSGGGGSDIVMTQSHKFMSTSVGDRVSIICKASQDVGTAVDWYQQKPGQSPKLLIYWASTRHTGVPDRFTGSGSGTDFTLTITNVQSEDLADYFCQQYNSYPLTFGAGTMLDLKRSDPAEPKSPDKTHTCPPCPAPPVAGPSVFLFPPKPKDTLMIARTPEVTCVVVDVSHEDPEVKFNWYVDGVEVHNAKTKPREEQYNSTYRVVSVLTVLHQDWLNGKEYKCKVSNKALPAPIEKTISKAKGQPREPQVYTLPPSRDELTKNQVSLTCLVKGFYPSDIAVEWESNGQPENNYKTTPPVLDSDGSFFLYSKLTVDKSRWQQGNVFSCSVMHEALHNHYTQKSLSLSPGKFWVLVVVGGVLACYSLLVTVAFIIFWVRRVKFSRSADAPAYQQGQNQLYNELNLGRREEYDVLDKRRGRDPEMGGKPRRKNPQEGLYNELQKDKMAEAYSEIGMKGERRRGKGHDGLYQGLSTATKDTYDALHMQALPPRRAEGRGSLLTCGDVEENPGPMETDTLILWVLLLLVPGSTGQVQLQQSGAELAKPGASVKMSCKTSGYSFSSYWMHWVKQRPGQGLEWIGYINPSTGYTENNQKFKDKVTLTADKSSNTAYMQLNSLTSEDSAVYYCARSGRLYFDVWGAGTTVTVSSGGGGSGGGGSGGGGSGGGGSDIVLTQSPPSLAVSLGQRATISCRASESIDLYGFTFMHWYQQKPGQPPKILIYRASNLESGIPARFSGSGSRTDFTLTINPVEADDVATYYCQQTHEDPYTFGGGTKLEIKSDPATTTPAPRPPTPAPTIASQPLSLRPEACRPAAGGAVHTRGLDFACDIVVISVGSMGLIISLLCVYFWLERTMPRIPTLKNLEDLVTEYHGNFSAWSGVSKGLAESLQPDYSERLCLVSEIPPKGGALGEGPGASPCNQHSPYWAPPCYTLKPETQCTNYALLKLAGDVESNPGPMETDTLILWVLLLLVPGSTGQVQLQQSGPELVKPGASVKISCKVSGYAISSSWMNWVKQRPGQGLEWIGRIYPGDGDTKYNGKFKDKATLTVDKSSSTAYMQLSSLTSVDSAVYFCARDGYRYYFDYWGQGTSVTVSSGGGGSGGGGSGGGGSGGGGSDIVMTQTAPSVFVTPGESVSISCRSSKSLLHSNGNTYLYWFLQRPGQSPQLLIYRMSNLASGVPDRFSGSGSGTDFTLRISRVEAEDVGVYYCMQHLEYPVTFGAGTKVEIKSDPAKIEVMYPPPYLDNEKSNGTIIHVKGKHLCPSPLFPGPSKPIPWLGHLLVGLSGAFGFIILVYLLINCRNTGPWLKKVLKCNTPDPSKFFSQLSSEHGGDVQKWLSSPFPSSSFSPGGLAPEISPLEVLERDKVTQLLLQQDKVPEPASLSSNHSLTSCFTNQGYFFFHLPDALEIEACQVYFTYDPYSEEDPDEGVAGAPTGSSPQPLQPLSGEDDAYCTFPSRDDLLLFSPSLLGGPSPPSTAPGGSGAGEERMPPSLQERVPRDWDPQPLGPPTPGVPDLVDFQPPPELVLREAGEEVPDAGPREGVSFPWSRPPGQGEFRALNARLPLNTDAYLSLQELQGQDPTHLV

SEQ ID NO: 46 - protein, 1631 aa, Artificial Sequence
  fusion construct with IL-7R alpha chain
MSLPVTALLLPLALLLHAAEVQLQQSGPELKKPGTSVRISCKTSGYTFTEYTIHWVKQSHGKSLEWIGNINPNNGGTTYNQKFEDKATLTVDKSSSTAYMELRSLTSEDSAVYYCAAGWNFDYWGQGTTLTVSSGGGGSGGGGSGGGGSDIVMTQSHKFMSTSVGDRVSIICKASQDVGTAVDWYQQKPGQSPKLLIYWASTRHTGVPDRFTGSGSGTDFTLTITNVQSEDLADYFCQQYNSYPLTFGAGTMLDLKRSDPAEPKSPDKTHTCPPCPAPPVAGPSVFLFPPKPKDTLMIARTPEVTCVVVDVSHEDPEVKFNWYVDGVEVHNAKTKPREEQYNSTYRVVSVLTVLHQDWLNGKEYKCKVSNKALPAPIEKTISKAKGQPREPQVYTLPPSRDELTKNQVSLTCLVKGFYPSDIAVEWESNGQPENNYKTTPPVLDSDGSFFLYSKLTVDKSRWQQGNVFSCSVMHEALHNHYTQKSLSLSPGKFWVLVVVGGVLACYSLLVTVAFIIFWVRRVKFSRSADAPAYQQGQNQLYNELNLGRREEYDVLDKRRGRDPEMGGKPRRKNPQEGLYNELQKDKMAEAYSEIGMKGERRRGKGHDGLYQGLSTATKDTYDALHMQALPPRRAEGRGSLLTCGDVEENPGPMETDTLILWVLLLLVPGSTGQVQLQQSGAELAKPGASVKMSCKTSGYSFSSYWMHWVKQRPGQGLEWIGYINPSTGYTENNQKFKDKVTLTADKSSNTAYMQLNSLTSEDSAVYYCARSGRLYFDVWGAGTTVTVSSGGGGSGGGGSGGGGSGGGGSDIVLTQSPPSLAVSLGQRATISCRASESIDLYGFTFMHWYQQKPGQPPKILIYRASNLESGIPARFSGSGSRTDFTLTINPVEADDVATYYCQQTHEDPYTFGGGTKLEIKSDPATTTPAPRPPTPAPTIASQPLSLRPEACRPAAGGAVHTRGLDFACDIVVISVGSMGLIISLLCVYFWLERTMPRIPTLKNLEDLVTEYHGNFSAWSGVSKGLAESLQPDYSERLCLVSEIPPKGGALGEGPGASPCNQHSPYWAPPCYTLKPETQCTNYALLKLAGDVESNPGPMETDTLILWVLLLLVPGSTGQVQLQQSGPELVKPGASVKISCKVSGYAISSSWMNWVKQRPGQGLEWIGRIYPGDGDTKYNGKFKDKATLTVDKSSSTAYMQLSSLTSVDSAVYFCARDGYRYYFDYWGQGTSVTVSSGGGGSGGGGSGGGGSGGGGSDIVMTQTAPSVFVTPGESVSISCRSSKSLLHSNGNTYLYWFLQRPGQSPQLLIYRMSNLASGVPDRFSGSGSGTDFTLRISRVEAEDVGVYYCMQHLEYPVTFGAGTKVEIKSDPAKIEVMYPPPYLDNEKSNGTIIHVKGKHLCPSPLFPGPSKPPILLTISILSFFSVALLVILACVLWKKRIKPIVWPSLPDHKKTLEHLCKKPRKNLNVSFNPESFLDCQIHRVDDIQARDEVEGFLQDTFPQQLEESEKQRLGGDVQSPNCPSEDVVITPESFGRDSSLTCLAGNVSACDAPILSSSRSLDCRESGKNGPHVYQDLLLSLGTTNSTLPPPFSLQSGILTLNPVAQGQPILTSLGSNQEEAYVTMSSFYQNQ

SEQ ID NO: 47 - protein, 19 aa, Artificial Sequence
  signal sequence derived from human CD8a
MSLPVTALLLPLALLLHAA

SEQ ID NO: 48 - protein, 4 aa, Artificial Sequence
  linker
SDPA

SEQ ID NO: 49 - protein, 231 aa, Artificial Sequence
  human IgG1Fc spacer (HCH2CH3pvaa)
EPKSPDKTHTCPPCPAPPVAGPSVFLFPPKPKDTLMIARTPEVTCVVVDVSHEDPEVKFNWYVDGVEVHNAKTKPREEQYNSTYRVVSVLTVLHQDWLNGKEYKCKVSNKALPAPIEKTISKAKGQPREPQVYTLPPSRDELTKNQVSLTCLVKGFYPSDIAVEWESNGQPENNYKTTPPVLDSDGSFFLYSKLTVDKSRWQQGNVFSCSVMHEALHNHYTQKSLSLSPGK

SEQ ID NO: 50 - protein, 27 aa, Artificial Sequence
  transmembrane derived from human CD28
FWVLVVVGGVLACYSLLVTVAFIIFWV

SEQ ID NO: 51 - protein, 113 aa, Artificial Sequence
  endodomain derived from TCRz
RRVKFSRSADAPAYQQGQNQLYNELNLGRREEYDVLDKRRGRDPEMGGKPRRKNPQEGLYNELQKDKMAEAYSEIGMKGERRRGKGHDGLYQGLSTATKDTYDALHMQALPPR

SEQ ID NO: 52 - protein, 20 aa, Artificial Sequence
  signal sequence derived from mouse kappa VIII
METDTLILWVLLLLVPGSTG

SEQ ID NO: 53 - protein, 40 aa, Artificial Sequence
  human CD28STK spacer
KIEVMYPPPYLDNEKSNGTIIHVKGKHLCPSPLFPGPSKP

SEQ ID NO: 54 - protein, 4 aa, Artificial Sequence
  furin cleavage site
  misc_feature (2)..(2): Xaa can be any naturally occurring amino acid
  MISC_FEATURE (3)..(3): Xaa can be Arg or Lys
RXXR

SEQ ID NO: 55 - protein, 7 aa, Artificial Sequence
  consensus Tobacco Etch Virus (TEV) cleavage site
ENLYFQS